European Patent Specification EP 3 784 686 B9, published October 4, 2023. Title: Rubella Virus Spike Konstrukt. Applicant: Institut Virion Serion GmbH. The sequence listing filed with the application follows.

SEQUENCE LISTING (8 sequences)

SEQ ID NO: 1 - DNA, 2112 bp, Rubella virus
ggactgcagccacgcgctgatatggctgctccaccaatgccaccacagccaccacgtgctcacggacagcactacggacaccaccatcaccagctgccatttctgggccacgatggacatcatggcggaacactgcgtgtgggacagcatcaccgtaacgccagtgatgtgctgccaggccattggttgcaaggcggatggggctgctacaacctgagcgattggcaccagggaacccacgtgtgccacaccaagcacatggatttttggtgcgtggaacacgatcgcccgccaccagctacaccaaccagtctgacaacagccgccaatagcaccactgccgctacaccagcaacagccccaccaccatgtcacgccggactgaatgatagctgcggcggatttctgagcggctgcggaccaatgcgtctgcgccatggtgctgatacacgttgcggacgcctgatttgcggcctgagtaccaccgctcagtacccaccaacacgcttcggatgcgctatgcgttggggactgccaccatgggaactcgtggtgttgacagcccgtccagaggatggatggacatgtcgcggagtgccagctcatccaggcacacgttgtccagaactggtgtccccaatgggacgtgccacatgtagtccagccagtgccttgtggctggccacagccaatgctttgagtggcggaagtggtggctcaggcggatcaggtggtggaagtggcggaggatctggaagcggaggcggtggcggagaagaggcctttacctacttgtgcacagccccaggatgcgccacacagacacctgtgccagttcgtctggctggcgtgcgcttcgagagcaagattgtggatggcggatgcttcgccccgtgggatctcgaagctactggtgcctgcatctgcgagatccccacagatgtgtcctgcgaaggactcggagcttgggtgccaacagctccatgcgctcgcatttggaatggaacccagcgcgcctgcacattctgggccgtgaatgcttatagcagcggcggctatgcccagctggcctcctactttaatccaggcggcagctactacaagcagtaccatccaaccgcctgcgaggtggaaccagccttcggacatagtgatgccgcctgctggggattcccaaccgatacagtgatgagcgtgttcgccctggccagctacgtgcagcatccacataagaccgtgcgcgtgaagttccacaccgagacacgtacagtgtggcagttgagtgtggccggcgtgtcctgcaatgtgaccaccgaacatccgttctgcaacaccccacacggccagttggaagtgcaagtgccaccagatccaggcgatctggtcgagtacatcatgaactacaccggcaaccagcagagccgctggggactgggaagcccaaattgccatggaccggattgggcaagcccagtgtgccaacgtcatagcccagattgcagtcgcctcgtgggagccacaccagaacgtccacgtctgcgtttggtggatgccgatgatccactgctgcgtactgctccaggaccaggcgaagtgtgggttaccccagtgattggaagccaggctcgcaagtgcggcctgcatattcgtgccggaccatacggacatgccaccgtggaaatgcccgagtggattcacgcccacaccaccagcgatccatggcacccaccaggaccactgggcctgaagtttaagacagtgcgcccagtggccttgccacgagctttggctccaccacgtaatgtgcgagtgaccggctgctaccagtgcggaacaccagctctggtggaaggattggctcccggcggaggcaattgtcacctgacagtgaatggcgaggatgtgggcgctttcccaccgggcaaatttgtgacagccgccttgctgaataccccgccaccttaccaagtgtcgtgcggcggagaaagtgatcgtgctagcgcccgtgtgatcgatccagctgctcagagttttaccggcgtggtgtacggcacccataccacagccgttagtgaaacccgtcagacctgggccgaatgggctgctgctcat

SEQ ID NO: 2 - protein, 722 aa, Rubella virus
MKLCILLAVVAFVGLSLGGLQPRADMAAPPMPPQPPRAHGQHYGHHHHQLPFLGHDGHHGGTLRVGQHHRNASDVLPGHWLQGGWGCYNLSDWHQGTHVCHTKHMDFWCVEHDRPPPATPTSLTTAANSTTAATPATAPPPCHAGLNDSCGGFLSGCGPMRLRHGADTRCGRLICGLSTTAQYPPTRFGCAMRWGLPPWELVVLTARPEDGWTCRGVPAHPGTRCPELVSPMGRATCSPASALWLATANALSGGSGGSGGSGGGSGGGSGSGGGGGEEAFTYLCTAPGCATQTPVPVRLAGVRFESKIVDGGCFAPWDLEATGACICEIPTDVSCEGLGAWVPTAPCARIWNGTQRACTFWAVNAYSSGGYAQLASYFNPGGSYYKQYHPTACEVEPAFGHSDAACWGFPTDTVMSVFALASYVQHPHKTVRVKFHTETRTVWQLSVAGVSCNVTTEHPFCNTPHGQLEVQVPPDPGDLVEYIMNYTGNQQSRWGLGSPNCHGPDWASPVCQRHSPDCSRLVGATPERPRLRLVDADDPLLRTAPGPGEVWVTPVIGSQARKCGLHIRAGPYGHATVEMPEWIHAHTTSDPWHPPGPLGLKFKTVRPVALPRALAPPRNVRVTGCYQCGTPALVEGLAPGGGNCHLTVNGEDVGAFPPGKFVTAALLNTPPPYQVSCGGESDRASARVIDPAAQSFTGVVYGTHTTAVSETRQTWAEWAAAH

SEQ ID NO: 3 - DNA, 2064 bp, Rubella virus
ggactgcagccacgcgctgatatggctgctccaccaatgccaccacagccaccacgtgctcacggacagcactacggacaccaccatcaccagctgccatttctgggccacgatggacatcatggcggaacactgcgtgtgggacagcatcaccgtaacgccagtgatgtgctgccaggccattggttgcaaggcggatggggctgctacaacctgagcgattggcaccagggaacccacgtgtgccacaccaagcacatggatttttggtgcgtggaacacgatcgcccgccaccagctacaccaaccagtctgacaacagccgccaatagcaccactgccgctacaccagcaacagccccaccaccatgtcacgccggactgaatgatagctgcggcggatttctgagcggctgcggaccaatgcgtctgcgccatggtgctgatacacgttgcggacgcctgatttgcggcctgagtaccaccgctcagtacccaccaacacgcttcggatgcgctatgcgttggggactgccaccatgggaactcgtggtgttgacagcccgtccagaggatggatggacatgtcgcggagtgccagctcatccaggcacacgttgtccagaactggtgtccccaatgggacgtgccacatgtagtccagccagtgccttgtggctggccacagccaatgctttgagtggcggaagtggtggctcaggcggagaagaggcctttacctacttgtgcacagccccaggatgcgccacacagacacctgtgccagttcgtctggctggcgtgcgcttcgagagcaagattgtggatggcggatgcttcgccccgtgggatctcgaagctactggtgcctgcatctgcgagatccccacagatgtgtcctgcgaaggactcggagcttgggtgccaacagctccatgcgctcgcatttggaatggaacccagcgcgcctgcacattctgggccgtgaatgcttatagcagcggcggctatgcccagctggcctcctactttaatccaggcggcagctactacaagcagtaccatccaaccgcctgcgaggtggaaccagccttcggacatagtgatgccgcctgctggggattcccaaccgatacagtgatgagcgtgttcgccctggccagctacgtgcagcatccacataagaccgtgcgcgtgaagttccacaccgagacacgtacagtgtggcagttgagtgtggccggcgtgtcctgcaatgtgaccaccgaacatccgttctgcaacaccccacacggccagttggaagtgcaagtgccaccagatccaggcgatctggtcgagtacatcatgaactacaccggcaaccagcagagccgctggggactgggaagcccaaattgccatggaccggattgggcaagcccagtgtgccaacgtcatagcccagattgcagtcgcctcgtgggagccacaccagaacgtccacgtctgcgtttggtggatgccgatgatccactgctgcgtactgctccaggaccaggcgaagtgtgggttaccccagtgattggaagccaggctcgcaagtgcggcctgcatattcgtgccggaccatacggacatgccaccgtggaaatgcccgagtggattcacgcccacaccaccagcgatccatggcacccaccaggaccactgggcctgaagtttaagacagtgcgcccagtggccttgccacgagctttggctccaccacgtaatgtgcgagtgaccggctgctaccagtgcggaacaccagctctggtggaaggattggctcccggcggaggcaattgtcacctgacagtgaatggcgaggatgtgggcgctttcccaccgggcaaatttgtgacagccgccttgctgaataccccgccaccttaccaagtgtcgtgcggcggagaaagtgatcgtgctagcgcccgtgtgatcgatccagctgctcagagttttaccggcgtggtgtacggcacccataccacagccgttagtgaaacccgtcagacctgggccgaatgggctgctgctcat

SEQ ID NO: 4 - protein, 706 aa, Rubella virus
MKLCILLAVVAFVGLSLGGLQPRADMAAPPMPPQPPRAHGQHYGHHHHQLPFLGHDGHHGGTLRVGQHHRNASDVLPGHWLQGGWGCYNLSDWHQGTHVCHTKHMDFWCVEHDRPPPATPTSLTTAANSTTAATPATAPPPCHAGLNDSCGGFLSGCGPMRLRHGADTRCGRLICGLSTTAQYPPTRFGCAMRWGLPPWELVVLTARPEDGWTCRGVPAHPGTRCPELVSPMGRATCSPASALWLATANALSGGSGGSGGEEAFTYLCTAPGCATQTPVPVRLAGVRFESKIVDGGCFAPWDLEATGACICEIPTDVSCEGLGAWVPTAPCARIWNGTQRACTFWAVNAYSSGGYAQLASYFNPGGSYYKQYHPTACEVEPAFGHSDAACWGFPTDTVMSVFALASYVQHPHKTVRVKFHTETRTVWQLSVAGVSCNVTTEHPFCNTPHGQLEVQVPPDPGDLVEYIMNYTGNQQSRWGLGSPNCHGPDWASPVCQRHSPDCSRLVGATPERPRLRLVDADDPLLRTAPGPGEVWVTPVIGSQARKCGLHIRAGPYGHATVEMPEWIHAHTTSDPWHPPGPLGLKFKTVRPVALPRALAPPRNVRVTGCYQCGTPALVEGLAPGGGNCHLTVNGEDVGAFPPGKFVTAALLNTPPPYQVSCGGESDRASARVIDPAAQSFTGVVYGTHTTAVSETRQTWAEWAAAH

SEQ ID NO: 5 - DNA, 1338 bp, Rubella virus
gaagaggcctttacctacttgtgcacagccccaggatgcgccacacagacacctgtgccagttcgtctggctggcgtgcgcttcgagagcaagattgtggatggcggatgcttcgccccgtgggatctcgaagctactggtgcctgcatctgcgagatccccacagatgtgtcctgcgaaggactcggagcttgggtgccaacagctccatgcgctcgcatttggaatggaacccagcgcgcctgcacattctgggccgtgaatgcttatagcagcggcggctatgcccagctggcctcctactttaatccaggcggcagctactacaagcagtaccatccaaccgcctgcgaggtggaaccagccttcggacatagtgatgccgcctgctggggattcccaaccgatacagtgatgagcgtgttcgccctggccagctacgtgcagcatccacataagaccgtgcgcgtgaagttccacaccgagacacgtacagtgtggcagttgagtgtggccggcgtgtcctgcaatgtgaccaccgaacatccgttctgcaacaccccacacggccagttggaagtgcaagtgccaccagatccaggcgatctggtcgagtacatcatgaactacaccggcaaccagcagagccgctggggactgggaagcccaaattgccatggaccggattgggcaagcccagtgtgccaacgtcatagcccagattgcagtcgcctcgtgggagccacaccagaacgtccacgtctgcgtttggtggatgccgatgatccactgctgcgtactgctccaggaccaggcgaagtgtgggttaccccagtgattggaagccaggctcgcaagtgcggcctgcatattcgtgccggaccatacggacatgccaccgtggaaatgcccgagtggattcacgcccacaccaccagcgatccatggcacccaccaggaccactgggcctgaagtttaagacagtgcgcccagtggccttgccacgagctttggctccaccacgtaatgtgcgagtgaccggctgctaccagtgcggaacaccagctctggtggaaggattggctcccggcggaggcaattgtcacctgacagtgaatggcgaggatgtgggcgctttcccaccgggcaaatttgtgacagccgccttgctgaataccccgccaccttaccaagtgtcgtgcggcggagaaagtgatcgtgctagcgcccgtgtgatcgatccagctgctcagagttttaccggcgtggtgtacggcacccataccacagccgttagtgaaacccgtcagacctgggccgaatgggctgctgctcat

SEQ ID NO: 6 - protein, 446 aa, Rubella virus
EEAFTYLCTAPGCATQTPVPVRLAGVRFESKIVDGGCFAPWDLEATGACICEIPTDVSCEGLGAWVPTAPCARIWNGTQRACTFWAVNAYSSGGYAQLASYFNPGGSYYKQYHPTACEVEPAFGHSDAACWGFPTDTVMSVFALASYVQHPHKTVRVKFHTETRTVWQLSVAGVSCNVTTEHPFCNTPHGQLEVQVPPDPGDLVEYIMNYTGNQQSRWGLGSPNCHGPDWASPVCQRHSPDCSRLVGATPERPRLRLVDADDPLLRTAPGPGEVWVTPVIGSQARKCGLHIRAGPYGHATVEMPEWIHAHTTSDPWHPPGPLGLKFKTVRPVALPRALAPPRNVRVTGCYQCGTPALVEGLAPGGGNCHLTVNGEDVGAFPPGKFVTAALLNTPPPYQVSCGGESDRASARVIDPAAQSFTGVVYGTHTTAVSETRQTWAEWAAAH

SEQ ID NO: 7 - DNA, 702 bp, Rubella virus
ggactgcagccacgcgctgatatggctgctccaccaatgccaccacagccaccacgtgctcacggacagcactacggacaccaccatcaccagctgccatttctgggccacgatggacatcatggcggaacactgcgtgtgggacagcatcaccgtaacgccagtgatgtgctgccaggccattggttgcaaggcggatggggctgctacaacctgagcgattggcaccagggaacccacgtgtgccacaccaagcacatggatttttggtgcgtggaacacgatcgcccgccaccagctacaccaaccagtctgacaacagccgccaatagcaccactgccgctacaccagcaacagccccaccaccatgtcacgccggactgaatgatagctgcggcggatttctgagcggctgcggaccaatgcgtctgcgccatggtgctgatacacgttgcggacgcctgatttgcggcctgagtaccaccgctcagtacccaccaacacgcttcggatgcgctatgcgttggggactgccaccatgggaactcgtggtgttgacagcccgtccagaggatggatggacatgtcgcggagtgccagctcatccaggcacacgttgtccagaactggtgtccccaatgggacgtgccacatgtagtccagccagtgccttgtggctggccacagccaatgctttgagt

SEQ ID NO: 8 - protein, 234 aa, Rubella virus
GLQPRADMAAPPMPPQPPRAHGQHYGHHHHQLPFLGHDGHHGGTLRVGQHHRNASDVLPGHWLQGGWGCYNLSDWHQGTHVCHTKHMDFWCVEHDRPPPATPTSLTTAANSTTAATPATAPPPCHAGLNDSCGGFLSGCGPMRLRHGADTRCGRLICGLSTTAQYPPTRFGCAMRWGLPPWELVVLTARPEDGWTCRGVPAHPGTRCPELVSPMGRATCSPASALWLATANALS